European Patent Specification EP 3 322 433 B1, published May 31, 2023. Title: Novel proteins specific for LAG-3. Applicant: Pieris AG. The sequence listing filed with the application follows.

SEQUENCE LISTING (58 sequences)

SEQ ID NO: 1 - protein, 158 aa, Homo sapiens
  Human tear lipocalin
HHLLASDEEIQDVSGTWYLKAMTVDREFPEMNLESVTPMTLTTLEGGNLEAKVTMLISGRCQEVKAVLEKTDEPGKYTADGGKHVAYIIRSHVKDHYIFYCEGELHGKPVRGVKLVGRDPKNNLEALEDFEKAAGARGLSTESILIPRQSETCSPGSD

SEQ ID NO: 2 - protein, 676 aa, Artificial Sequence
  Fusion protein of Cynomolgus LAG-3 extracellular domain and IgG1 Fc
PQPGAEISVVWAQEGAPAQLPCSPTIPLQDLSLLRRAGVTWQHQPDSGPPAPAPGHPPVPGHRPAAPYSWGPRPRRYTVLSVGPGGLRSGRLPLQPRVQLDERGRQRGDFSLWLRPARRADAGEYRATVHLRDRALSCRLRLRVGQASMTASPPGSLRTSDWVILNCSFSRPDRPASVHWFRSRGQGRVPVQGSPHHHLAESFLFLPHVGPMDSGLWGCILTYRDGFNVSIMYNLTVLGLEPATPLTVYAGAGSRVELPCRLPPAVGTQSFLTAKWAPPGGGPDLLVAGDNGDFTLRLEDVSQAQAGTYICHIRLQGQQLNATVTLAIITVTPKSFGSPGSLGKLLCEVTPASGQEHFVWSPLNTPSQRSFSGPWLEAQEAQLLSQPWQCQLHQGERLLGAAVYFTELSSPGAQRSGRAPGALRAGHLIEGRMDGGGGSGGGGSGGGGSDKTHTCPPCPAPELLGGPSVFLFPPKPKDTLMISRTPEVTCVVVDVSHEDPEVKFNWYVDGVEVHNAKTKPREEQYNSTYRVVSVLTVLHQDWLNGKEYKCKVSNKALPAPIEKTISKAKGQPREPQVYTLPPSREEMTKNQVSLTCLVKGFYPSDIAVEWESNGQPENNYKTTPPVLDSDGSFFLYSKLTVDKSRWQQGNVFSCSVMHEALHNHYTQKSLSLSPGK

SEQ ID NO: 3 - protein, 152 aa, Artificial Sequence
  negative control 4008wt
ASDEEIQDVSGTWYLKAMTVDRECPEMNLESVTPMTLTTLEGGNLEAKVTMLISGRSQEVKAVLEKTDEPGKYTADGGKHVAYIIRSHVKDHYIFYSEGECHGKPVPGVWLVGRDPKNNLEALEDFEKAAGARGLSTESILIPRQSETSSPG

SEQ ID NO: 4 - protein, 152 aa, Artificial Sequence
  negative control 4009wt
ASDEEIQDVPGTWYLKAMTVDREFPEMNLESVTPMTLTTLEGGNLEAKVTMLISGRCQEVKAVLEKTDEPGKYTADGGKHVAYIIRSHVKDHYIFYSEGELHGKPVRGVKLVGRDPTNNLEALEDFEKAAGARGLSTESILIPRQSETCSPG

SEQ ID NO: 5 - protein, 447 aa, Artificial Sequence
  benchmark antibody heavy chain
QVQLQQWGAGLLKPSETLSLTCAVYGGSFSDYYWNWIRQPPGKGLEWIGEINHRGSTNSNPSLKSRVTLSLDTSKNQFSLKLRSVTAADTAVYYCAFGYSDYEYNWFDPWGQGTLVTVSSASTKGPSVFPLAPCSRSTSESTAALGCLVKDYFPEPVTVSWNSGALTSGVHTFPAVLQSSGLYSLSSVVTVPSSSLGTKTYTCNVDHKPSNTKVDKRVESKYGPPCPPCPAPEFLGGPSVFLFPPKPKDTLMISRTPEVTCVVVDVSQEDPEVQFNWYVDGVEVHNAKTKPREEQFNSTYRVVSVLTVLHQDWLNGKEYKCKVSNKGLPSSIEKTISKAKGQPREPQVYTLPPSQEEMTKNQVSLTCLVKGFYPSDIAVEWESNGQPENNYKTTPPVLDSDGSFFLYSRLTVDKSRWQEGNVFSCSVMHEALHNHYTQKSLSLSLGK

SEQ ID NO: 6 - protein, 214 aa, Artificial Sequence
  benchmark antibody light chain
EIVLTQSPATLSLSPGERATLSCRASQSISSYLAWYQQKPGQAPRLLIYDASNRATGIPARFSGSGSGTDFTLTISSLEPEDFAVYYCQQRSNWPLTFGQGTNLEIKRTVAAPSVFIFPPSDEQLKSGTASVVCLLNNFYPREAKVQWKVDNALQSGNSQESVTEQDSKDSTYSLSSTLTLSKADYEKHKVYACEVTHQGLSSPVTKSFNRGEC

SEQ ID NO: 7 - protein, 152 aa, Artificial Sequence
  lipocalin mutein
ASDEEIQDVSGTWYLKAMTVDSDCFWIEEWSVTPMTLTTLEGGNLEAKVTMDIFGFWQEVKAVLEKTDEPGKYTADGGKHVAYIIRSHVKDHYIFYSEGECAGFPVPGVWLVGRDPKNNLEALEDFEKAAGARGLSTESILIPRQSETSSPG

SEQ ID NO: 8 - protein, 152 aa, Artificial Sequence
  lipocalin mutein
ASDEEIQDVPGTWYLKAMTVSGEDPEMTLESVTPMTLTTLEGGNLEANVTALIDGRCQEVKNVLEKTDEPGKYTEDGGKHVDYIIRSHVKDHYIFYFEGEGHGTPARTVALVGRDPTNNLEALEDFEKAAGARGLSTESILIPRQSETCSPG

SEQ ID NO: 9 - protein, 152 aa, Artificial Sequence
  lipocalin mutein
ASDEEIQDVSGTWYLKAMTVDFVCLYDVPESVTPMTLTTLEGGNLEAKVTMQIWGELQEVKAVLEKTDEPGKYTADGGKHVAYIIRSHVKDHYIFYSEGYCVGYPVPGVWLVGRDPKNNLEALEDFEKAAGARGLSTESILIPRQSETSSPG

SEQ ID NO: 10 - protein, 152 aa, Artificial Sequence
  lipocalin mutein
ASDEEIQDVSGTWYLKAMTVDETCWWYVDHSVTPMTLTTLEGGNLEAKVTMNLWGFWQEVKAVLEKTDEPGKYTADGGKHVAYIIRSHVKDHYIFYSEGECQGWPVPGVWLVGRDPKNNLEALEDFEKAAGARGLSTESILIPRQSETSSPG

SEQ ID NO: 11 - protein, 152 aa, Artificial Sequence
  lipocalin mutein
ASDEEIQDVSGTWYLKAMTVDSDCFWIDDVSVTPMTLTTLEGGNLEAKVTMDIFGFWQEVKAVLEKTDEPGKYTADGGKHVAYIIRSHVKDHYIFYSEGECAGYPVPGVWLVGRDPKNNLEALEDFEKAAGARGLSTESILIPRQSETSSPG

SEQ ID NO: 12 - protein, 152 aa, Artificial Sequence
  lipocalin mutein
ASDEEIQDVSGTWYLKAMTVDSDCFWIDEVSVTPMTLTTLEGGNLEAKVTMDIFGFWQEVKAVLEKTDEPGKYTADGGKHVAYIIRSHVKDHYIFYSEGECAGYPVPGVWLVGRDPKNNLEALEDFEKAAGARGLSTESILIPRQSETSSPG

SEQ ID NO: 13 - protein, 152 aa, Artificial Sequence
  lipocalin mutein
ASDEEIQDVSGTWYLKAMTVDSDCFWIEEWSATPMTLTTLEGGDLEAKVTMDIFGFWQEVKAVLEKTDEPGKYTADGGKHAAYIIRSHVKDHYIFYSEGECAGFPVPGVWLVGRDPKNNLEALEDFEKAAGARGLGTESILIPRQSETSSPG

SEQ ID NO: 14 - protein, 152 aa, Artificial Sequence
  lipocalin mutein
ASDEEIQDVSGTWYLKAMTVDSDCFWIDEVSVTPMTLTTLEGGNLEAKVTMDIFGFWQEVKAVLEKTDEPGKYTADGGKHVAYIIRSHVKDHYIFYSEGECEGFPVPGVWLVGRDPKNNLEALEDFEKAAGARGLSTESILIPRQSETSSPG

SEQ ID NO: 15 - protein, 152 aa, Artificial Sequence
  lipocalin mutein
ASDEEIQDVSGTWYLKAMTVDSDCFWIEEWSATPMTLTTLEGGNLEAEATMDIFGFWQEVKAVLEKTDEPGKYTADGGKHVAYIIRSHVKDHYIFYSEGECAGFPVPGVWLVGRDPKNNLEALEDFEKAAGARGLSTESILIPRQSETSSPG

SEQ ID NO: 16 - protein, 152 aa, Artificial Sequence
  lipocalin mutein
ASDEEIQDVSGTWYLKAMTVDSDCFWVDEVSVTPMTLTTLEGGNLEAKVTMDIFGFWQEVKAVLEKTDEPGKYTADGGKHVAYIIRSHVKDHYIFYSEGECAGFPVPGVWLVGRDPKNNLEALEDFEKAAGARGLSTESILIPRQSETSSPG

SEQ ID NO: 17 - protein, 152 aa, Artificial Sequence
  lipocalin mutein
ASDEEIQDVPGTWYLKAMTVSGEDPELWLESVTPMTLTTLEGGNLEASVTALIDGRCQEVKNVLEKTDEPGKYTEDGGKHVDYIIRSHVKDHYIFYFEGEGYGTPGRMVALVGRDPTNNLEALEDFEKAAGARGLSTESILIPRQSETCSPG

SEQ ID NO: 18 - protein, 152 aa, Artificial Sequence
  lipocalin mutein
ASDEEIQDVPGTWYLKAMTVSAEDPELVLESVTPMTLTTLEGGNLEASVTALIDGRCQEVKNVLEKTDEPGKYTEDGGKHVDYIIRSHVKDHYIFYFEGEGHGTPARTVALVGRDPTNNLEALEDFEKAAGARGLSTESILIPRQSETCSPG

SEQ ID NO: 19 - protein, 152 aa, Artificial Sequence
  lipocalin mutein
ASDEEIQDVPGTWYLKAMTVSDEDPEMTLESVTPMTLTTLEGGNLEASVTALIDGRCQEVKNVLEKTDEPGKYTEDGGKHVDYIIRSHVKDHYIFYFEGEGQGTPGRMVALVGRDPTNNLEALEDFEKAAGARGLSTESILIPRQSETCSPG

SEQ ID NO: 20 - protein, 152 aa, Artificial Sequence
  lipocalin mutein
ASDEEIQDVPGTWYLKAMTVSEEDPEMTLESVTPMTLTTLEGGNLEASVTALIDGRCQEVKNVLEKTDEPGKYTEDGGKHVDYIIRSHVKDHYIFYFEGEGHGTPGRMVALVGRDPTNNLEALEDFEKAAGARGLSTESILIPRQSETCSPG

SEQ ID NO: 21 - protein, 152 aa, Artificial Sequence
  lipocalin mutein
ASDEEIQDVPGTWYLKAMTVSGEDPEMMLESVTPMTLTTLEGGNLEARVTVLIDGRCQEVKNVLEKTDEPGKYTEDGGKHVDYIIRSHVKDHYIFYFEGEGQGTPGRMVALVGRDPTNNLEALEDFEKAAGARGLSTESILIPRQSETCSPG

SEQ ID NO: 22 - protein, 152 aa, Artificial Sequence
  lipocalin mutein
ASDEEIQDVSGTWYLKAMTVDFVCLNDYPESVTPMTLTTLEGGNLEAKVTMQIWGEPQEVKAVLEKTDEPGKYTADGGKHVAYIIRSHVKDHYIFYSEGYCTGYPVPGVWLVGRDPKNNLEALEDFEKAAGARGLSTESILIPRQSETSSPG

SEQ ID NO: 23 - DNA, 637 bp, Artificial Sequence
  lipocalin mutein
gcctcagacgaggagattcaggatgtgtcagggacgtggtatctgaaggccatgacggtggattctgattgtttttggatagaggagtggtcagttacgccaatgactctgactacccttgaaggcggcaatctggaggctaaggtcaccatggatatatttgggttctggcaggaggtgaaagcagtgttagagaagacagatgaaccgggtaaatatacggccgatggcggtaaacatgttgcctatatcattcgcagccatgtgaaagatcattacatcttttatagcgagggcgagtgcgcagggtttccggttccaggggtgtggctcgtgggcagagaccccaagaacaacctggaagccttggaggactttgagaaagccgcaggagcccgcggactcagcacggagagcatcctcatccccaggcagagcgaaaccagctctccagggagcgcttggtctcacccgcagttcgaaaaataataagcttgacctgtgaagtgaaaaatggcgcacattgtgcgacattttttttgtctgccgtttaccgctactgcgtcacggatctccacgcgccctgtagcggcgcattaagcgcggcgggtgtggtggttacgcgcagcgtgaccgc

SEQ ID NO: 24 - DNA, 637 bp, Artificial Sequence
  lipocalin mutein
gcctcagacgaggagattcaggatgtgccagggacgtggtatctgaaagcgatgacggtttctggggaagatcctgagatgactctggaatcagttacgccaatgactctgactacccttgaaggcggcaatctggaggctaacgtcaccgcactgatcgatgggcgctgtcaagaagtgaagaatgtgctcgagaagacagatgaaccgggtaaatacacggaggacggcggtaaacatgtggattatatcattagatctcatgtgaaagatcattacatcttctactttgagggcgaggggcatggcactccggcacgtactgtggcactggtgggcagagaccccaccaataatctggaagccttggaggactttgagaaagccgcaggagcccgcggactcagcacggagagcatcctcatccccaggcagagcgaaacctgctctccagggagcgcttggtctcacccgcagttcgaaaaataataagcttgacctgtgaagtgaaaaatggcgcacattgtgcgacattttttttgtctgccgtttaccgctactgcgtcacggatctccacgcgccctgtagcggcgcattaagcgcggcgggtgtggtggttacgcgcagcgtgaccgc

SEQ ID NO: 25 - DNA, 637 bp, Artificial Sequence
  lipocalin mutein
gcctcagacgaggagattcaggatgtgtcagggacgtggtatctgaaggccatgacggtggattttgtgtgtctgtatgatgtgcctgagtcagttacgccaatgactctgactacccttgaaggcggcaatctggaggctaaggtcaccatgcaaatatggggggagctgcaagaggtgaaagcagtgttagagaagacagatgaaccgggtaaatatacggccgatggcggtaaacatgttgcctatatcattcgcagccatgtgaaagatcattacatcttttatagcgagggctattgtgtggggtatcctgttccaggggtgtggctcgtgggcagagaccccaagaacaacctggaagccttggaggactttgagaaagccgcaggagcccgcggactcagcacggagagcatcctcatccccaggcagagcgaaaccagctctccagggagcgcttggtctcacccgcagttcgaaaaataataagcttgacctgtgaagtgaaaaatggcgcacattgtgcgacattttttttgtctgccgtttaccgctactgcgtcacggatctccacgcgccctgtagcggcgcattaagcgcggcgggtgtggtggttacgcgcagcgtgaccgc

SEQ ID NO: 26 - DNA, 456 bp, Artificial Sequence
  lipocalin mutein
gcctcagacgaggagattcaggatgtgtcagggacgtggtatctgaaggccatgacggtggatgagacttgttggtggtatgtggatcattcagttacgccaatgactctgactacccttgaaggcggcaatctggaggctaaggtcaccatgaatctctgggggttctggcaggaggtgaaagcagtgttagagaagacagatgaaccgggtaaatatacggccgatggcggtaaacatgttgcctatatcattcgcagccatgtgaaagatcattacatcttttatagcgagggagagtgccaagggtggccggttccaggggtgtggctcgtgggcagagaccccaagaacaacctggaagccttggaggactttgagaaagccgcaggagcccgcggactcagcacggagagcatcctcatccccaggcagagcgaaaccagctctccaggg

SEQ ID NO: 27 - DNA, 637 bp, Artificial Sequence
  lipocalin mutein
gcctcagacgaggagattcaggatgtgtcagggacgtggtatctgaaggccatgacggtggattctgattgcttttggattgatgatgtgtcagttacgccaatgactctgactacccttgaaggcggcaatctggaggctaaggtcaccatggatatttttggcttttggcaggaagtgaaagcagtgttagagaagacagatgaaccgggtaaatatacggccgatggcggcaaacatgttgcctatatcattcgcagccatgtgaaagatcattacatcttttatagcgagggcgaatgcgctggctatccggttccaggggtgtggctcgtgggcagagaccccaagaacaacctggaagccttggaggactttgagaaagccgcaggagcccgcggactcagcacggagagcatcctcatccccaggcagagcgaaaccagctctccagggagcgcttggtctcacccgcagttcgaaaaataataagcttgacctgtgaagtgaaaaatggcgcacattgtgcgacattttttttgtctgccgtttaccgctactgcgtcacggatctccacgcgccctgtagcggcgcattaagcgcggcgggtgtggtggttacgcgcagcgtgaccgc

SEQ ID NO: 28 - DNA, 637 bp, Artificial Sequence
  lipocalin mutein
gcctcagacgaggagattcaggatgtgtcagggacgtggtatctgaaggccatgacggtggattcggattgcttttggattgatgaggtgtcagttacgccaatgactctgactacccttgaaggcggcaatctggaggctaaggtcaccatggatatttttggcttttggcaggaagtgaaagcagtgttagagaagacagatgaaccgggtaaatatacggccgatggcggcaaacatgttgcctatatcattcgcagccatgtgaaagatcattacatcttttatagcgagggcgaatgcgctggctatccggttccaggggtgtggctcgtgggcagagaccccaagaacaacctggaagccttggaggactttgagaaagccgcaggagcccgcggactcagcacggagagcatcctcatccccaggcagagcgaaaccagctctccagggagcgcttggtctcacccgcagttcgaaaaataataagcttgacctgtgaagtgaaaaatggcgcacattgtgcgacattttttttgtctgccgtttaccgctactgcgtcacggatctccacgcgccctgtagcggcgcattaagcgcggcgggtgtggtggttacgcgcagcgtgaccgc

SEQ ID NO: 29 - DNA, 637 bp, Artificial Sequence
  lipocalin mutein
gcctcagacgaggagattcaggatgtgtcagggacgtggtatctgaaggcgatgacggtggattctgattgtttttggatagaggagtggtcagctacgccaatgactctgactacccttgaaggtggcgatctggaggctaaggtcaccatggatatattcgggttctggcaggaggtgaaagcagtgttagagaagacagatgaaccgggtaaatatacggccgatggcggtaaacatgctgcctatatcattcgcagccatgtgaaagatcattacatcttttatagcgagggcgagtgcgcagggtttccggtcccgggggtgtggctcgtgggcagagaccccaagaacaacctggaagccttggaggactttgagaaagccgcaggagcccgcggactcggcacggagagcatcctcatccccaggcagagcgaaaccagctctccagggccaagcgcttggtctcacccgcagttcgaaaaataataagcttgacctgtgaagtgaaaaatggcgcacattgtgcgacattttttttgtctgccgtttaccgctactgcgtcacggatctccacgcgccctgtagcggcgcattaagcgcggcgggtgtggtggttacgcgcagcgtgac

SEQ ID NO: 30 - DNA, 637 bp, Artificial Sequence
  lipocalin mutein
gcctcagacgaggagattcaggatgtgtcagggacgtggtatctgaaggccatgacggtggattcggattgcttttggattgatgaggtgtcagttacgccaatgactctgactacccttgaaggcggcaatctggaggctaaggtcaccatggatatttttggcttttggcaggaagtgaaagcagtgttagagaagacagatgaaccgggtaaatatacggccgatggcggcaaacatgttgcctatatcattcgcagccatgtgaaagatcattacatcttttatagcgagggcgaatgcgagggctttccggttccaggggtgtggctcgtgggcagagaccccaagaacaacctggaagccttggaggactttgagaaagccgcaggagcccgcggactcagcacggagagcatcctcatccccaggcagagcgaaaccagctctccagggagcgcttggtctcacccgcagttcgaaaaataataagcttgacctgtgaagtgaaaaatggcgcacattgtgcgacattttttttgtctgccgtttaccgctactgcgtcacggatctccacgcgccctgtagcggcgcattaagcgcggcgggtgtggtggttacgcgcagcgtgaccgc

SEQ ID NO: 31 - DNA, 637 bp, Artificial Sequence
  lipocalin mutein
gcctcagacgaggagattcaggatgtgtcagggacgtggtatctgaaggcgatgacggtggattctgattgtttttggatagaggagtggtcagctacgccaatgactctgactacccttgaaggcggcaatctggaggctgaggccaccatggatatatttgggttctggcaggaggtgaaagcagtgttggagaagacagacgaaccgggtaaatatacggccgatggcggtaaacatgttgcctatatcattcgcagccatgtgaaagatcattacatcttttatagcgagggcgagtgcgcagggtttccggtcccgggggtgtggctcgtgggcagagaccccaagaacaacctggaagccttggaggactttgagaaagccgcaggagcccgcggactcagcacggagagcatcctcatccccaggcagagcgaaaccagctctccagggccaagcgcttggtctcacccgcagttcgaaaaataataagcttgacctgtgaagtgaaaaatggcgcacattgtgcgacattttttttgtctgccgtttaccgctactgcgtcacggatctccacgcgccctgtagcggcgcattaagcgcggcgggtgtggtggttacgcgcagcgtgac

SEQ ID NO: 32 - DNA, 637 bp, Artificial Sequence
  lipocalin mutein
gcctcagacgaggagattcaggatgtgtcagggacgtggtatctgaaggccatgacggtggattcggattgcttttgggtggatgaggtgtcagttacgccaatgactctgactacccttgaaggcggcaatctggaggctaaggtcaccatggatatttttggcttttggcaggaagtgaaagcagtgttagagaagacagatgaaccgggtaaatatacggccgatggcggcaaacatgttgcctatatcattcgcagccatgtgaaagatcattacatcttttatagcgagggcgaatgcgctggctttccggttccaggggtgtggctcgtgggcagagaccccaagaacaacctggaagccttggaggactttgagaaagccgcaggagcccgcggactcagcacggagagcatcctcatccccaggcagagcgaaaccagctctccagggagcgcttggtctcacccgcagttcgaaaaataataagcttgacctgtgaagtgaaaaatggcgcacattgtgcgacattttttttgtctgccgtttaccgctactgcgtcacggatctccacgcgccctgtagcggcgcattaagcgcggcgggtgtggtggttacgcgcagcgtgaccgc

SEQ ID NO: 33 - DNA, 637 bp, Artificial Sequence
  lipocalin mutein
gcctcagacgaggagattcaggatgtgccagggacgtggtatctgaaagcgatgacggtttcgggggaagatcctgagttgtggctggaatcagttacgccaatgactctgactacccttgaaggcggcaatctggaggctagtgtgaccgctctgattgatggccgctgccaggaagtgaaaaatgtgctcgagaagacagatgaaccgggtaaatacacggaggatggcggcaaacatgtggattatatcattagatctcatgtgaaagatcattacatcttctactttgaaggcgaaggttatggcacgccgggtcgcatggtggctctggtgggcagagaccccaccaataatctggaagccttggaggactttgagaaagccgcaggagcccgcggactcagcacggagagcatcctcatccccaggcagagcgaaacctgctctccagggagcgcttggtctcacccgcagttcgaaaaataataagcttgacctgtgaagtgaaaaatggcgcacattgtgcgacattttttttgtctgccgtttaccgctactgcgtcacggatctccacgcgccctgtagcggcgcattaagcgcggcgggtgtggtggttacgcgcagcgtgaccgc

SEQ ID NO: 34 - DNA, 637 bp, Artificial Sequence
  lipocalin mutein
gcctcagacgaggagattcaggatgtgccagggacgtggtatctgaaagcgatgacggtttcggcggaagatcctgagttggtgctggaatcagttacgccaatgactctgactacccttgaaggcggcaatctggaggcttctgtgaccgcgctgattgatggccgctgccaggaagtgaaaaatgtgctcgagaagacagatgaaccgggtaaatacacggaggatggcggcaaacatgtggattatatcattagatctcatgtgaaagatcattacatcttctactttgaaggcgaaggtcatggcactccggctcgcacggtggctctggtgggcagagaccccaccaataatctggaagccttggaggactttgagaaagccgcaggagcccgcggactcagcacggagagcatcctcatccccaggcagagcgaaacctgctctccagggagcgcttggtctcacccgcagttcgaaaaataataagcttgacctgtgaagtgaaaaatggcgcacattgtgcgacattttttttgtctgccgtttaccgctactgcgtcacggatctccacgcgccctgtagcggcgcattaagcgcggcgggtgtggtggttacgcgcagcgtgaccgc

SEQ ID NO: 35 - DNA, 637 bp, Artificial Sequence
  lipocalin mutein
gcctcagacgaggagattcaggatgtgccagggacgtggtatctgaaagcgatgacggtttctgatgaagatcctgagatgacgctggaatcagttacgccaatgactctgactacccttgaaggcggcaatctggaggctagtgtgaccgcgctgattgatggccgctgccaggaagtgaaaaatgtgctcgagaagacagatgaaccgggtaaatacacggaggatggcggcaaacatgtggattatatcattagatctcatgtgaaagatcattacatcttctactttgaaggcgaaggtcagggcacgccgggtcgcatggtggctctggtgggcagagaccccaccaataatctggaagccttggaggactttgagaaagccgcaggagcccgcggactcagcacggagagcatcctcatccccaggcagagcgaaacctgctctccagggagcgcttggtctcacccgcagttcgaaaaataataagcttgacctgtgaagtgaaaaatggcgcacattgtgcgacattttttttgtctgccgtttaccgctactgcgtcacggatctccacgcgccctgtagcggcgcattaagcgcggcgggtgtggtggttacgcgcagcgtgaccgc

SEQ ID NO: 36 - DNA, 637 bp, Artificial Sequence
  lipocalin mutein
gcctcagacgaggagattcaggatgtgccagggacgtggtatctgaaagcgatgacggtttctgaggaagatcctgagatgacgctggaatcagttacgccaatgactctgactacccttgaaggcggcaatctggaggctagtgtgaccgctctgattgatggccgctgccaggaagtgaaaaatgtgctcgagaagacagatgaaccgggtaaatacacggaggatggcggcaaacatgtggattatatcattagatctcatgtgaaagatcattacatcttctactttgaaggcgaaggtcatggcacgccgggtcgcatggtggctctggtgggcagagaccccaccaataatctggaagccttggaggactttgagaaagccgcaggagcccgcggactcagcacggagagcatcctcatccccaggcagagcgaaacctgctctccagggagcgcttggtctcacccgcagttcgaaaaataataagcttgacctgtgaagtgaaaaatggcgcacattgtgcgacattttttttgtctgccgtttaccgctactgcgtcacggatctccacgcgccctgtagcggcgcattaagcgcggcgggtgtggtggttacgcgcagcgtgaccgc

SEQ ID NO: 37 - DNA, 637 bp, Artificial Sequence
  lipocalin mutein
gcctcagacgaggagattcaggatgtgccagggacgtggtatctgaaagcgatgacggtttcgggggaagatcctgagatgatgctggaatcagttacgccaatgactctgactacccttgaaggcggcaatctggaggctcgtgtgaccgttctgattgatggccgctgccaggaagtgaaaaatgtgctcgagaagacagatgaaccgggtaaatacacggaggatggcggcaaacatgtggattatatcattagatctcatgtgaaagatcattacatcttctactttgaaggcgaagggcagggcacgccgggtcgcatggtggctctggtgggcagagaccccaccaataatctggaagccttggaggactttgagaaagccgcaggagcccgcggactcagcacggagagcatcctcatccccaggcagagcgaaacctgctctccagggagcgcttggtctcacccgcagttcgaaaaataataagcttgacctgtgaagtgaaaaatggcgcacattgtgcgacattttttttgtctgccgtttaccgctactgcgtcacggatctccacgcgccctgtagcggcgcattaagcgcggcgggtgtggtggttacgcgcagcgtgaccgc

SEQ ID NO: 38 - DNA, 637 bp, Artificial Sequence
  lipocalin mutein
gcctcagacgaggagattcaggatgtgtcagggacgtggtatctgaaggccatgacggtggattttgtgtgcctgaatgattatcctgagtcagttacgccaatgactctgactacccttgaaggcggcaatctggaggctaaggtcaccatgcagatttggggcgagccgcaggaagtgaaagcagtgttagagaagacagatgaaccgggtaaatatacggccgatggcggcaaacatgttgcctatatcattcgcagccatgtgaaagatcattacatcttttatagcgagggctattgcacgggctatccggttccaggggtgtggctcgtgggcagagaccccaagaacaacctggaagccttggaggactttgagaaagccgcaggagcccgcggactcagcacggagagcatcctcatccccaggcagagcgaaaccagctctccagggagcgcttggtctcacccgcagttcgaaaaataataagcttgacctgtgaagtgaaaaatggcgcacattgtgcgacattttttttgtctgccgtttaccgctactgcgtcacggatctccacgcgccctgtagcggcgcattaagcgcggcgggtgtggtggttacgcgcagcgtgaccgc

SEQ ID NO: 39 - DNA, 456 bp, Artificial Sequence
  lipocalin mutein
gcctcagacgaggagattcaggatgtgtcagggacgtggtatctgaaggccatgacggtggattctgattgtttttggatagaggagtggtcagttacgccaatgactctgactacccttgaaggcggcaatctggaggctaaggtcaccatggatatatttgggttctggcaggaggtgaaagcagtgttagagaagacagatgaaccgggtaaatatacggccgatggcggtaaacatgttgcctatatcattcgcagccatgtgaaagatcattacatcttttatagcgagggcgagtgcgcagggtttccggttccaggggtgtggctcgtgggcagagaccccaagaacaacctggaagccttggaggactttgagaaagccgcaggagcccgcggactcagcacggagagcatcctcatccccaggcagagcgaaaccagctctccaggg

SEQ ID NO: 40 - DNA, 456 bp, Artificial Sequence
  lipocalin mutein
gcctcagacgaggagattcaggatgtgccagggacgtggtatctgaaagcgatgacggtttctggggaagatcctgagatgactctggaatcagttacgccaatgactctgactacccttgaaggcggcaatctggaggctaacgtcaccgcactgatcgatgggcgctgtcaagaagtgaagaatgtgctcgagaagacagatgaaccgggtaaatacacggaggacggcggtaaacatgtggattatatcattagatctcatgtgaaagatcattacatcttctactttgagggcgaggggcatggcactccggcacgtactgtggcactggtgggcagagaccccaccaataatctggaagccttggaggactttgagaaagccgcaggagcccgcggactcagcacggagagcatcctcatccccaggcagagcgaaacctgctctccaggg

SEQ ID NO: 41 - DNA, 456 bp, Artificial Sequence
  lipocalin mutein
gcctcagacgaggagattcaggatgtgtcagggacgtggtatctgaaggccatgacggtggattttgtgtgtctgtatgatgtgcctgagtcagttacgccaatgactctgactacccttgaaggcggcaatctggaggctaaggtcaccatgcaaatatggggggagctgcaagaggtgaaagcagtgttagagaagacagatgaaccgggtaaatatacggccgatggcggtaaacatgttgcctatatcattcgcagccatgtgaaagatcattacatcttttatagcgagggctattgtgtggggtatcctgttccaggggtgtggctcgtgggcagagaccccaagaacaacctggaagccttggaggactttgagaaagccgcaggagcccgcggactcagcacggagagcatcctcatccccaggcagagcgaaaccagctctccaggg

SEQ ID NO: 42 - DNA, 456 bp, Artificial Sequence; identical to SEQ ID NO: 26
  lipocalin mutein

SEQ ID NO: 43 - DNA, 456 bp, Artificial Sequence
  lipocalin mutein
gcctcagacgaggagattcaggatgtgtcagggacgtggtatctgaaggccatgacggtggattctgattgcttttggattgatgatgtgtcagttacgccaatgactctgactacccttgaaggcggcaatctggaggctaaggtcaccatggatatttttggcttttggcaggaagtgaaagcagtgttagagaagacagatgaaccgggtaaatatacggccgatggcggcaaacatgttgcctatatcattcgcagccatgtgaaagatcattacatcttttatagcgagggcgaatgcgctggctatccggttccaggggtgtggctcgtgggcagagaccccaagaacaacctggaagccttggaggactttgagaaagccgcaggagcccgcggactcagcacggagagcatcctcatccccaggcagagcgaaaccagctctccaggg

SEQ ID NO: 44 - DNA, 456 bp, Artificial Sequence
  lipocalin mutein
gcctcagacgaggagattcaggatgtgtcagggacgtggtatctgaaggccatgacggtggattcggattgcttttggattgatgaggtgtcagttacgccaatgactctgactacccttgaaggcggcaatctggaggctaaggtcaccatggatatttttggcttttggcaggaagtgaaagcagtgttagagaagacagatgaaccgggtaaatatacggccgatggcggcaaacatgttgcctatatcattcgcagccatgtgaaagatcattacatcttttatagcgagggcgaatgcgctggctatccggttccaggggtgtggctcgtgggcagagaccccaagaacaacctggaagccttggaggactttgagaaagccgcaggagcccgcggactcagcacggagagcatcctcatccccaggcagagcgaaaccagctctccaggg

SEQ ID NO: 45 - DNA, 456 bp, Artificial Sequence
  lipocalin mutein
gcctcagacgaggagattcaggatgtgtcagggacgtggtatctgaaggcgatgacggtggattctgattgtttttggatagaggagtggtcagctacgccaatgactctgactacccttgaaggtggcgatctggaggctaaggtcaccatggatatattcgggttctggcaggaggtgaaagcagtgttagagaagacagatgaaccgggtaaatatacggccgatggcggtaaacatgctgcctatatcattcgcagccatgtgaaagatcattacatcttttatagcgagggcgagtgcgcagggtttccggtcccgggggtgtggctcgtgggcagagaccccaagaacaacctggaagccttggaggactttgagaaagccgcaggagcccgcggactcggcacggagagcatcctcatccccaggcagagcgaaaccagctctccaggg

SEQ ID NO: 46 - DNA, 456 bp, Artificial Sequence
  lipocalin mutein
gcctcagacgaggagattcaggatgtgtcagggacgtggtatctgaaggccatgacggtggattcggattgcttttggattgatgaggtgtcagttacgccaatgactctgactacccttgaaggcggcaatctggaggctaaggtcaccatggatatttttggcttttggcaggaagtgaaagcagtgttagagaagacagatgaaccgggtaaatatacggccgatggcggcaaacatgttgcctatatcattcgcagccatgtgaaagatcattacatcttttatagcgagggcgaatgcgagggctttccggttccaggggtgtggctcgtgggcagagaccccaagaacaacctggaagccttggaggactttgagaaagccgcaggagcccgcggactcagcacggagagcatcctcatccccaggcagagcgaaaccagctctccaggg

SEQ ID NO: 47 - DNA, 456 bp, Artificial Sequence
  lipocalin mutein
gcctcagacgaggagattcaggatgtgtcagggacgtggtatctgaaggcgatgacggtggattctgattgtttttggatagaggagtggtcagctacgccaatgactctgactacccttgaaggcggcaatctggaggctgaggccaccatggatatatttgggttctggcaggaggtgaaagcagtgttggagaagacagacgaaccgggtaaatatacggccgatggcggtaaacatgttgcctatatcattcgcagccatgtgaaagatcattacatcttttatagcgagggcgagtgcgcagggtttccggtcccgggggtgtggctcgtgggcagagaccccaagaacaacctggaagccttggaggactttgagaaagccgcaggagcccgcggactcagcacggagagcatcctcatccccaggcagagcgaaaccagctctccaggg

SEQ ID NO: 48 - DNA, 456 bp, Artificial Sequence
  lipocalin mutein
gcctcagacgaggagattcaggatgtgtcagggacgtggtatctgaaggccatgacggtggattcggattgcttttgggtggatgaggtgtcagttacgccaatgactctgactacccttgaaggcggcaatctggaggctaaggtcaccatggatatttttggcttttggcaggaagtgaaagcagtgttagagaagacagatgaaccgggtaaatatacggccgatggcggcaaacatgttgcctatatcattcgcagccatgtgaaagatcattacatcttttatagcgagggcgaatgcgctggctttccggttccaggggtgtggctcgtgggcagagaccccaagaacaacctggaagccttggaggactttgagaaagccgcaggagcccgcggactcagcacggagagcatcctcatccccaggcagagcgaaaccagctctccaggg

SEQ ID NO: 49 - DNA, 456 bp, Artificial Sequence
  lipocalin mutein
gcctcagacgaggagattcaggatgtgccagggacgtggtatctgaaagcgatgacggtttcgggggaagatcctgagttgtggctggaatcagttacgccaatgactctgactacccttgaaggcggcaatctggaggctagtgtgaccgctctgattgatggccgctgccaggaagtgaaaaatgtgctcgagaagacagatgaaccgggtaaatacacggaggatggcggcaaacatgtggattatatcattagatctcatgtgaaagatcattacatcttctactttgaaggcgaaggttatggcacgccgggtcgcatggtggctctggtgggcagagaccccaccaataatctggaagccttggaggactttgagaaagccgcaggagcccgcggactcagcacggagagcatcctcatccccaggcagagcgaaacctgctctccaggg

SEQ ID NO: 50 - DNA, 456 bp, Artificial Sequence
  lipocalin mutein
gcctcagacgaggagattcaggatgtgccagggacgtggtatctgaaagcgatgacggtttcggcggaagatcctgagttggtgctggaatcagttacgccaatgactctgactacccttgaaggcggcaatctggaggcttctgtgaccgcgctgattgatggccgctgccaggaagtgaaaaatgtgctcgagaagacagatgaaccgggtaaatacacggaggatggcggcaaacatgtggattatatcattagatctcatgtgaaagatcattacatcttctactttgaaggcgaaggtcatggcactccggctcgcacggtggctctggtgggcagagaccccaccaataatctggaagccttggaggactttgagaaagccgcaggagcccgcggactcagcacggagagcatcctcatccccaggcagagcgaaacctgctctccaggg

SEQ ID NO: 51 - DNA, 456 bp, Artificial Sequence
  lipocalin mutein
gcctcagacgaggagattcaggatgtgccagggacgtggtatctgaaagcgatgacggtttctgatgaagatcctgagatgacgctggaatcagttacgccaatgactctgactacccttgaaggcggcaatctggaggctagtgtgaccgcgctgattgatggccgctgccaggaagtgaaaaatgtgctcgagaagacagatgaaccgggtaaatacacggaggatggcggcaaacatgtggattatatcattagatctcatgtgaaagatcattacatcttctactttgaaggcgaaggtcagggcacgccgggtcgcatggtggctctggtgggcagagaccccaccaataatctggaagccttggaggactttgagaaagccgcaggagcccgcggactcagcacggagagcatcctcatccccaggcagagcgaaacctgctctccaggg

SEQ ID NO: 52 - DNA, 456 bp, Artificial Sequence
  lipocalin mutein
gcctcagacgaggagattcaggatgtgccagggacgtggtatctgaaagcgatgacggtttctgaggaagatcctgagatgacgctggaatcagttacgccaatgactctgactacccttgaaggcggcaatctggaggctagtgtgaccgctctgattgatggccgctgccaggaagtgaaaaatgtgctcgagaagacagatgaaccgggtaaatacacggaggatggcggcaaacatgtggattatatcattagatctcatgtgaaagatcattacatcttctactttgaaggcgaaggtcatggcacgccgggtcgcatggtggctctggtgggcagagaccccaccaataatctggaagccttggaggactttgagaaagccgcaggagcccgcggactcagcacggagagcatcctcatccccaggcagagcgaaacctgctctccaggg

SEQ ID NO: 53 - DNA, 456 bp, Artificial Sequence
  lipocalin mutein
gcctcagacgaggagattcaggatgtgccagggacgtggtatctgaaagcgatgacggtttcgggggaagatcctgagatgatgctggaatcagttacgccaatgactctgactacccttgaaggcggcaatctggaggctcgtgtgaccgttctgattgatggccgctgccaggaagtgaaaaatgtgctcgagaagacagatgaaccgggtaaatacacggaggatggcggcaaacatgtggattatatcattagatctcatgtgaaagatcattacatcttctactttgaaggcgaagggcagggcacgccgggtcgcatggtggctctggtgggcagagaccccaccaataatctggaagccttggaggactttgagaaagccgcaggagcccgcggactcagcacggagagcatcctcatccccaggcagagcgaaacctgctctccaggg

SEQ ID NO: 54 - DNA, 456 bp, Artificial Sequence
  lipocalin mutein
gcctcagacgaggagattcaggatgtgtcagggacgtggtatctgaaggccatgacggtggattttgtgtgcctgaatgattatcctgagtcagttacgccaatgactctgactacccttgaaggcggcaatctggaggctaaggtcaccatgcagatttggggcgagccgcaggaagtgaaagcagtgttagagaagacagatgaaccgggtaaatatacggccgatggcggcaaacatgttgcctatatcattcgcagccatgtgaaagatcattacatcttttatagcgagggctattgcacgggctatccggttccaggggtgtggctcgtgggcagagaccccaagaacaacctggaagccttggaggactttgagaaagccgcaggagcccgcggactcagcacggagagcatcctcatccccaggcagagcgaaaccagctctccaggg

SEQ ID NO: 55 - protein, 4 aa, Homo sapiens
  N-terminal sequence of human tear lipocalin
HHLL

SEQ ID NO: 56 - protein, 4 aa, Artificial sequence
  Factor Xa cleavage site
IEGR

SEQ ID NO: 57 - protein, 10 aa, Artificial Sequence
  SA linker and strep-tag II fusion peptide
SAWSHPQFEK

SEQ ID NO: 58 - protein, 8 aa, Artificial Sequence
  Strep-tag II peptide
WSHPQFEK